European Patent Specification EP 3 600 375 B1, published November 5, 2025. Title: Bacteriocins for control of Salmonella enterica. Applicant: Nomad Bioscience GmbH. The sequence listing filed with the application follows.

SEQUENCE LISTING (24 sequences)

SEQ ID NO: 1 - protein, 583 aa, Salmonella enterica
MSGGDGIGHNSGAHSTGGVNGSSSGRGGSSSGGGNNPNSGPGWGTTHTPDGHDIHNYNPGEFGGGGHKPGGNGGNHSGGTGDGQPPGAAMAFGFPALVPAGAGGLAVTVSGDALAAAIADVLAVLKGPFKFGAWGIALYGILPTEIAKDDPRMMSKIVTSLPADAVTESPVSSLPLDQATVSVTKRVTDVVKDERQHIAVVAGVPASIPVVDAKPTTHPGVFSVSVPGLPDLQVSTVKNAPAMTALPRGVTDEKDRTVHPAGFTFGGSSHEAVIRFPKESGQAPVYVSVTDVLTPEQVKQRQDEENRRQQEWDATHPVEVAERNYRLASDELNRANVDVAGKQERQIQAAQAVAARKGELDAANKTFADAKEEIKKFERFAHDPMAGGHRMWQMAGLKAQRAQNEVNQKQAEFNAAEKEKADADAALNVALESRKQKEQKAKDASDKLDKENKRNHPGKATGKGQPVGDKWLEDAGKEAGAPVPDRIADKLRDKEFKNFDDFRKKFWEEVSKDPELSKQFIPGNKKRMSQGLAPRARNKDTVGGRRSFELHHDKPISQDGGVYDMDNIRVTTPKLHIDIHRGK

SEQ ID NO: 2 - protein, 587 aa, Salmonella enterica
MSGGDGRGHNTGAHSTSGNINGGPTGLGVSGGASDGSGWSSENNPWGGGSGSGIHWGGGSGRGNGGGNGNSGGGSGTGGNLSAVAAPVAFGFPALSTPGAGGLAVSISASELSAAIAGIIAKLKKVNLKFTPFGVVLSSLIPSEIAKDDPNMMSKIVTSLPADDITESPVSSLPLDKATVNVNVRVVDDVKDERQNISVVSGVPMSVPVVDAKPTERPGVFTASIPGAPVLNISVNNSTPAVQTLSPGVTNNTDKDVRPAGFTQGGNTRDAVIRFPKDSGHNAVYVSVSDVLSPDQVKQRQDEENRRQQEWDATHPVEVAEREYENARAELEAENKNVHSLQVALDGLKNTAEGLALSDAGRHPLTSSESRFVAVPGYSGGGVHFDATATVDSRDRLNSLLSLGGAAYVNNVLELGEVSAPTEDGLKVGNAIKNAMIEVYDKLRQRLITRQNEINHAQVSLNTAIESRNKKEEKKRSAENKLNEERNKPRKGTKDYGHDYHPAPETEEIKGLGDIKKGIPKTPKQNGGGKRKRWIGDKGRKIYEWDSQHGELEGYRASDGQHLGSFDPKTGKQLKGPDPKRNIKKYL

SEQ ID NO: 3 - protein, 585 aa, Salmonella enterica
MSGGDGIGHNSGAHSTGGVNGSSSGSGGSSSGSGNNPNSGPGWGTTHTPNGDIHNYNPGEFGGGGNKPGGHGGNSGNHDGSSGNGQPSAAPMAFGFPALAPAGAGSLAVTVSGEALSAAIADIFAALKGPFKFGAWGIALYGIMPTEIAKDDPNMMSKIMTSLPADTVTDTPVSSLPLDQATVSVTKRVADVVKDERQHIAVVAGVPMSVPVVDAKPTTRPGIFSATVPGLPALEVSTGKSIPASTALPRGITEDKDRTEHPAGFTFGGSSHDAVIRFPKESGQAPVYVSVTDVLTPEQVKQRQDEESRRQQEWDATHPVEVAERNYRLASDELNRVNADVAGKQERQAQAGQAVAARKGELDAANKTFADAKEEIKKFEHFARDPMAGGHRMWQMAGLKAQRAQNEVNQKQAEFDAAEKEKADADAALNAALESRKQKEQKAKDTKERLDKENKRNQPGKATGKGQPVSDKWLEDAGKESGSPIPDSIADKLRDKEFRNFDDFRKKFWEEVSKDPELSKQFIKGNRDRMQVGKAPKSRKKDAAGKRTSFELHHDKPVSQDGGVYDMDNLRITTPKRHIDIHRGQ

SEQ ID NO: 4 - protein, 483 aa, Salmonella enterica
MADNTIAYYEDGVPHSADGKVVIVIDGKMPVDTGAGGTGGGGGGKVGGTSESSAAIHATAKWSTAQLKKTLAEKAARERETAAAMAAAKAKRDALTQHLKDIVNDVLRHNASRTPSATDLAHANNMAMQAEAQRLGRAKAEEKARKEAEAAELAFQEAERQREEAVRQLAETERQLKQAEEEKRLAALSDEARAVENARKNLDTAKSELANVDSDIERQRSQLSSLDADVKKAEENLRLTMRIKGRIGRKMQAKSQAIVDDKKRIYSDAENVLNTMTVNRNLKAQQVTDAENELKVAIDNLNSSQMKNAVDATVSFYQTLTEKYGEKYSLIAQELAEKSKGKKIGNVDEALAAFEKYKDVLDKKFSKADRDAIVNALKSFNYDDWAKHLDQFAKYLKITGHVSFGYDVVSDVLKASETGDWKPLFITLEQKVLDTGMSYLVVLMFSLIAGTTLGIFGVAIITAILCSFVDKYILNALNDALGI

SEQ ID NO: 5 - protein, 527 aa, Salmonella enterica
MSDNTIAYYEDGVPYSADGQVVIVIDGKMPVDTGAGGTGGGGGGKVGGTSESSAAIHATAKWSKAQLQKSLEEKAARERETAAAMAAAKAKRDALTQHLKDIVNDVLRYNASRTPSATDLAHANNMAMQAEAQRLGRAKAEEKARKEAEAAEKSLQEAERQREEAARQRAEAERQLKQAEAEEKRLAALSEEARAVEITQKNLAAAQSELSKMDGEIKSLNVRLSTSIHARDAEMNSLSGKRNELAQESAKYKELDELVKKLEPRANDPLQNRPFFDATSRRARAGDTLAEKQKEVTASETRINELNTEINQVRGAISQANNNRNLKVQQVTETENALKVAIDNLNSSQMKNAVDATVSFYQTLTAKYGEKYSLIAQELAEQSKGKKISNVDEALAAFEKYKDVLDKKFSKADRDAIVNALKSVDYADWAKHLDQFSRYLKISGRVSTGYDIYSDIRKGMDTNDWRPLFLTLEKLAVDAGVGYIVALGFSVIASTALGIWGVAIITGVICSFVDKKDLEKLNEALGI

SEQ ID NO: 6 - protein, 296 aa, Salmonella enterica
MFIKSGGNLTIRTFGGLGVGGDFDSDTWRRRSTDSWVPYSEYIAIECIVAPNQLYQLLTDVAQVETVAAQLAQVGYQYLQGRLRLVREDGSCTDFSGKAMLDNLLNKSKDILDLDFLHVSEGYRSEAYWPGQSSGITIGYGVDIGHQSEEGLHKWGVPQSIIDKIKDYFGITGEAANTLLKGLKDKTLGLSDREIKQFSDIVKKQATADIINKYNAATKGITFDKIPYNTRTAIIDLFYQYSAPKGAPKSWGFIINNDWNGFYNELMNFGDKHTTRREREAALVLSDIVNNQYIYK

SEQ ID NO: 7 - protein, 100 aa, Salmonella enterica
MELKKSISDYTEAEFKKIIEAIINCEGDEKTQDDNLEFFIRVTEYPSGSDLIYYPEGDNDGSTEAIIKEIKEWRAANGKPGFKQADSSYFVSFDYRDGDW

SEQ ID NO: 8 - protein, 87 aa, Salmonella enterica
MELKNSISDYTEAEFIEFMKEIDKENVAETDDKLDLLLNHFEQVTEHPDGTDLIYYAASDAESTPEAITKKIKEWRAANGKPGFKQG

SEQ ID NO: 9 - protein, 499 aa, Escherichia coli
MAKELSVYGPTAGESMGGTGANLNQQGGNNNSNSGVHWGGGSGSGNGGREHGSQTGWGWSKTNNPDVPPYVDDNGQVRITITNGLVKTPVYGVPGAGGNSDVQGGYIPENPNDEVARKWDKNNLPREIDVSIDGFKYRVTLNDNGRAIGILRTGVRPYVGSEKAKAGIMEKINHKTPEEIYEALGFNKDESQRQEKAKQQAEDAWDRLPPNVRKFDVDVEQFHYLVVLDDYGNVLSVTRTGVRPYVGSEKAKAGIMDKVDHKTPEEIYEALGFNNEEPQRQNQAKKAAYDVFYSFSMNRDRIQSDVLNKAAEVISDIGNKVGDYLGDAYKSLAREIADDVKNFQGKTIRSYDDAMASLNKVLSNPGFKFNRADSDALANVWRSIDAQDMANKLGNISKAFKFADVVMKVEKVREKSIEGYETGNWGPLMLEVESWVLSGIASAVALGVFSATLGAYALSLGAPAIAVGIVGILLAAVVGALLDDKFADALNKEIIKPAH

SEQ ID NO: 10 - protein, 490 aa, Escherichia coli
MDKVTDNSPDVESTESTEGSFPTVGVDTGDTITATLATGTENVGGGGGAFGGASESSAAIHATAKWSTAQLKKHQAEQAARAAAAEAALAKAKSQRDALTQRLKDIVNDALRANAARSPSVTDLAHANNMAMQAEAERLRLAKAEQKAREEAEAAEKALREAERQRDEIARQQAETAHLLAMAEAAEAEKNRQDSLDEEHRAVEVAEKKLAEAKAELAKAESDVQSKQAIVSRVAGELENAQKSVDVKVTGFPGWRDVQKKLERQLQDKKNEYSSVTNALNSAVSIRDAKKTDVQNAEIKLKEAKDALEKSQVKDSVDTMVGFYQYITEQYGEKYSRIAQDLAEKAKGSKFSSVDEALAAFEKYKNVLDKKISKVDRDAIFNALESVNYDELSKNLTKISKSLKITSRVSFLYDVGSDFKNAIETGNWRPLFVTLEKSAVDVGVAKIVALMFSFIVGVPLGFWGIAIVTGIVSSYIGDDELNKLNELLGI

SEQ ID NO: 11 - protein, 490 aa, Escherichia coli
MDKVTDNSPDVESTESTEGSFPTVGVDTGDTITATLATGTENVGGGGGAFGGASESSAAIHATAKWSTAQLKKHQAEQAARAAAAEAALAKAKSQRDALTQRLKDIVNDALRANAARSPSVTDLAHANNMAMQAEAERLRLAKAEQKAREEAEAAEKALREAERQRDEIARQQAETAHLLAMAEAAEAEKNRQDSLDEEHRAVEVAEKKLAEAKAELAKAESDVQSKQAIVSRVAGELENAQKSVDVKVTGFPGWRDVQKKLERQLQDKKNEYSSVTNALNSAVSIRDAKKTEVQNAEIKLKEAKDALEKSQVKDSVDTMVGFYQYITEQYGEKYSRIAQDLAEKAKGSKFNSVDEALAAFEKYKNVLDKKFSKVDRDDIFNALESITYDEWAKHLEKISRALKVTGYLSFGYDVWDGTLKGLKTGDWKPLFVTLEKSAVDFGVAKIVALMFSFIVGAPLGFWGIAIITGIVSSYIGDDELNKLNELLGI

SEQ ID NO: 12 - protein, 626 aa, Escherichia coli
MSDPVRITNPGAESLGYDSDGHEIMAVDIYVNPPRVDVFHGTPPAWSSFGNKTIWGGNEWVDDSPTRSDIEKRDKEITAYKNTLSAQQKENENKRTEAGKRLSAAIAAREKDENTLKTLRAGNADAADITRQEFRLLQAELREYGFRTEIAGYDALRLHTESRMLFADADSLRISPREARSLIEQAEKRQKDAQNADKKAADMLAEYERRKGILDTRLSELEKNGGAALAVLDAQQARLLGQQTRNDRAISEARNKLSSVTESLNTARNALTRAEQQLTQQKNTPDGKTIVSPEKFPGRSSTNHSIVVSGDPRFAGTIKITTSAVIDNRANLNYLLTHSGLDYKRNILNDRNPVVTEDVEGDKKIYNAEVAEWDKLRQRLLDARNKITSAESAVNSARNNLSARTNEQKHANDALNALLKEKENIRNQLAGINQKIAEEKRKQDELKATKDAINFTTEFLKSVSEKYGAKAEQLAREMAGQAKGKKIRNVEEALKTYEKYRADINKKINAKDRAAIAAALESVKLSDISSNLNRFSRGLGYAGKFTSLADWITEFGKAVRTENWRPLFVKTETIIAGNAATALVALVFSILTGSALGIIGYGLLMAVTGALIDESLVEKANKFWGI

SEQ ID NO: 13 - protein, 626 aa, Escherichia coli
MSDPVRITNPGAESLGYDSDGHEIMAVDIYVNPPRVDVFHGTPPAWSSFGNKTIWGGNEWVDDSPTRSDIEKRDKEITAYKNTLSAQQKENENKRTEAGKRLSAAIAAREKDENTLKTLRAGNADAADITRQEFRLLQAELREYGFRTEIAGYDALRLHTESRMLFADADSLRISPREARSLIEQAEKRQKDAQNADKKAADMLAEYERRKGILDTRLSELEKNGGAALAVLDAQQARLLGQQTRNDRAISEARNKLSSVTESLKTARNALTRAEQQLTQQKNTPDGKTIVSPEKFPGRSSTNHSIVVSGDPRFAGTIKITTSAVIDNRANLNYLLTHSGLDYKRNILNDRNPVVTEDVEGDKKIYNAEVAEWDKLRQRLLDARNKITSAESAINSARNNVSARTNEQKHANDALNALLKEKENIRSQLADINQKIAEEKRKRDEINMVKDAIKLTSDFYRTIYDEFGKQASELAKELASVSQGKQIKSVDDALNAFDKFRNNLNKKYNIQDRMAISKALEAINQVHMAENFKLFSKAFGFTGKVIERYDVAVELQKAVKTDNWRPFFVKLESLAAGRAASAVTAWAFSVMLGTPVGILGFAIIMAAVSALVNDKFIEQVNKLIGI

SEQ ID NO: 14 - protein, 271 aa, Escherichia coli
METLTVHAPSPSTNLPSYGNGAFSLSAPHVPGAGPLLVQVVYSFFQSPNMCLQALTQLEDYIKKHGASNPLTLQIISTNIGYFCNADRNLVLHPGISVYDAYHFAKPAPSQYDYRSMNMKQMSGNVTTPIVALAHYLWGNGAERSVNIANIGLKISPMKINQIKDIIKSGVVGTFPVSTKFTHATGDYNVITGAYLGNITLKTEGTLTISANGSWTYNGVVRSYDDKYDFNASTHRGIIGESLTRLGAMFSGKEYQILLPGEIHIKESGKR

SEQ ID NO: 15 - DNA, 1942 bp, Artificial Sequence
  codon-optimized sequence for expressing ScolE2
atgtctggtggtgatggtatcggtcacaatagcggtgctcattctactggtggtgtgaacggttcttcatctggtaggggtggtagttcttcaggtggtggtaacaaccctaactctggtcctggttggggtactactcatactcctgatggtcacgatatccacaactacaaccctggtgagtttggtggtggtggacataagcctggtggaaacggtggtaatcactctggtggtactggtgatggacaacctcctggtgctgctatggcttttggtttccctgctcttgttcctgctggtgctggtggtcttgctgttactgtttctggtgatgctctggctgctgcaattgctgatgtgcttgctgttctgaagggacctttcaagtttggtgcttggggtatcgctctgtacggtattcttcctaccgagatcgctaaggatgatccaaggatgatgagcaagatcgtgacctctttgcctgctgatgctgtgactgagtctcctgtgtcatctctgcctcttgatcaggctactgtgagcgttaccaagagggttaccgatgtggttaaggatgagaggcagcacattgctgttgttgctggtgtgcctgcttctatccctgttgttgatgctaagcctactacccaccctggtgtgttctctgtttctgttcctggtctgcctgatctgcaggtttcaactgtgaagaacgctcctgctatgactgctttgcctaggggtgttactgatgagaaggataggactgttcaccctgctggtttcaccttcggtggttcttctcatgaggctgtgatcaggttccctaaagagtctggtcaggctcctgtttacgtgtcagtgaccgatgttcttacccctgagcaggttaagcagagacaggatgaagagaatagaaggcagcaagagtgggatgctactcaccctgttgaagtggctgagaggaattacaggctggcttctgatgagctgaacagggctaatgtggatgtggctggtaagcaagagaggcagattcaagctgctcaagctgttgctgctagaaagggtgaactggatgctgctaacaagaccttcgctgatgctaaagaagagatcaagaagttcgagaggttcgctcacgatcctatggctggtggacacagaatgtggcaaatggctggtcttaaggctcagagggctcagaatgaggttaaccagaaacaagctgagttcaacgctgctgagaaagaaaaggctgatgcagatgctgctctgaacgtggcacttgagtctaggaagcagaaagaacaaaaggcaaaggatgctagcgataagctggataaggaaaacaagaggaaccaccctggaaaggctactggtaagggtcaacctgttggtgataagtggcttgaggatgctggtaaagaagctggagcacctgttccagataggatcgctgataagctgagagataaggaattcaagaacttcgatgattttaggaagaagttctgggaagaggtaaatttctagtttttctccttcattttcttggttaggacccttttctctttttatttttttgagctttgatctttctttaaactgatctattttttaattgattggttatggtgtaaatattacatagctttaactgataatctgattactttatttcgtgtgtctatgatgatgatgataactgcaggttagcaaggatcctgagctgagcaagcagttcatccctggtaacaagaaaaggatgagccagggtcttgctcctagggctagaaacaaggatactgtgggtggtagaagatccttcgagctgcatcacgataagccaatctctcaggatggtggtgtttacgatatggataacatcagggtgaccaccccaaagctgcacatcgatattcataggggaaagtaa

SEQ ID NO: 16 - DNA, 1954 bp, Artificial Sequence
  codon-optimized coding sequence for expressing ScolE3
atgtctggtggtgatggtaggggtcataataccggtgctcatagcaccagcggtaacattaacggtggtcctactggtcttggtgtgtcaggtggtgcttctgatggttctggttggtcctctgagaacaatccttggggtggtggtagcggttctggtattcactggggaggtggaagtggtagaggtaatggtggtggaaacggtaacagtggtggtggttctggaactggtggtaacctttctgctgttgctgctcctgttgctttcggtttccctgctctttctactcctggtgctggtggtttggctgtgtctatttctgcttctgagctgagcgctgctatcgctggtattatcgctaagctgaagaaggtgaacctgaagttcacccctttcggtgtggtgctgtcctctttgattcctagcgagatcgctaaggatgatcctaacatgatgagcaagatcgtgaccagcctgcctgctgatgatattaccgagtctcctgtgtcctctctgcctcttgataaggctactgtgaatgtgaacgtgagggtggtggatgatgtgaaggatgagaggcagaacatcagcgttgtgtctggtgttcctatgtctgtgcctgttgtggatgctaagcctactgaaaggcctggtgtgttcaccgcttctattccaggtgctcctgtgctgaacatctccgtgaacaattctacccctgctgtgcagactctttctcctggtgtgactaacaacaccgataaggatgttaggcctgctggtttcactcagggtggtaataccagggatgctgtgatcaggttccctaaggattctggtcacaacgcagtgtacgtgtccgtgtctgatgtgttgtctccagatcaggttaagcagaggcaggatgaagagaatagaaggcagcaagagtgggatgctactcaccctgttgaagttgctgagagagagtacgagaacgctagagctgaacttgaggctgaaaacaagaacgtgcacagccttcaggtggcacttgatggtcttaagaataccgctgagggtctggctctttctgatgctggtagacatcctctgaccagcagcgagtctagatttgttgctgtgcctggttactccggtggtggtgttcattttgatgctaccgctaccgtggatagcagggataggcttaactctcttctgtctcttggtggtgctgcttacgtgaacaacgtgttggagcttggtgaggtgtcagctcctactgaggatggtttgaaggtgggaaacgctatcaagaacgctatgatcgaggtgtacgataagctgaggcagaggcttattaccaggcagaacgagatcaaccacgctcaggtgtcacttaacaccgctatcgagtctaggaacaagaaagaggaaaagaagaggtccgcagagaacaagctgaacgaagagagaaacaagcctagaaagggtactaaggattacggacacgattaccatcctgctccagagactgaagaaatcaagggtctgggtgatatcaagaagggtatccctaagacccctaagcagaacggtggtggtaagagaaagagatggatcggagataagggtagaaagatctacgagtgggatagccagcatggtgagcttgaaggtaaatttctagtttttctccttcattttcttggttaggacccttttctctttttatttttttgagctttgatctttctttaaactgatctattttttaattgattggttatggtgtaaatattacatagctttaactgataatctgattactttatttcgtgtgtctatgatgatgatgataactgcaggttatagggcttcagatggtcagcacctgggaagctttgatcctaagactggtaagcagctgaagggtcctgatccaaagaggaacatcaagaagtacctttaa

SEQ ID NO: 17 - DNA, 1948 bp, Artificial Sequence
  codon-optimized coding sequence for expressing ScolE7
atgtctggtggtgatggtatcggtcacaatagcggtgctcattctactggtggtgtgaacggttcctcttctggttctggtggaagctcatctggaagcggtaacaaccctaattctggtcctggttggggtactactcatacccctaacggtgatatccacaactacaaccctggtgagtttggtggtggtggaaacaagcctggtggacatggtggtaactctggtaaccacgatggtagctctggaaacggtcaaccttctgctgctcctatggcttttggtttccctgctcttgctcctgctggtgctggttctcttgctgttactgtttctggtgaggctctgtctgctgctatcgctgatattttcgctgctctgaagggacctttcaagttcggtgcttggggtattgctctgtacggtattatgcctaccgagatcgctaaggatgatcctaacatgatgagcaagatcatgaccagcctgcctgctgatactgtgactgatactcctgtgtcctctctgcctcttgatcaggctactgtgtctgtgactaagagggttgcagatgtggtgaaggatgagaggcagcatattgctgttgttgctggtgtgcctatgtctgtgcctgttgttgatgctaagcctaccactaggcctggtatcttctctgctactgttcctggacttcctgctttggaggtgtcaaccggtaagtctattcctgcttctaccgctctgcctaggggtattactgaggataaggataggactgagcaccctgctggtttcactttcggtggttcttctcacgatgctgtgatcaggttccctaaagagtctggtcaggctccagtttacgtgtcagtgactgatgtgcttacccctgagcaggttaagcagagacaggatgaagagtctagaaggcagcaagagtgggatgctactcatcctgttgaagtggctgagaggaactacaggcttgcttctgatgagctgaacagggtgaacgctgatgtggctggtaagcaagaaagacaagctcaagctggacaggctgttgctgctagaaagggtgaacttgatgctgctaacaagaccttcgctgatgctaaagaagagatcaagaagttcgagcacttcgctagggatccaatggctggtggtcatagaatgtggcagatggctggtcttaaggctcagagggctcagaatgaggttaaccagaaacaagctgagttcgatgctgcagagaaagaaaaggctgatgctgatgcagctctgaacgctgctcttgaatctaggaagcagaaagagcagaaggctaaggataccaaagagaggctggataaggaaaacaagaggaatcagcctggtaaggctaccggtaagggtcagccagtttctgataagtggcttgaggatgctggtaaagagagcggttctcctatccctgatagcattgctgataagcttagagataaggaattcagaaacttcgatgattttaggaagaagttctgggaggaagttagcaaggatcctgagctgagcaagcagttcatcaagggtaacagagataggatgcaggtaaatttctagtttttctccttcattttcttggttaggacccttttctctttttatttttttgagctttgatctttctttaaactgatctattttttaattgattggttatggtgtaaatattacatagctttaactgataatctgattactttatttcgtgtgtctatgatgatgatgataactgcaggttggaaaggctcctaagtccagaaagaaggatgctgctggtaagaggacctctttcgagcttcatcacgataagcctgtgagccaggatggtggtgtttacgatatggataacctgaggatcaccacccctaagaggcacatcgatattcataggggacagtaa

SEQ ID NO: 18 - DNA, 1452 bp, Artificial Sequence
  codon-optimized coding sequence for expressing ScolE1a
atggctgataacaccattgcttactacgaggatggtgtgcctcacagcgctgatggtaaggtggtgattgtgatcgatggtaagatgcctgtggataccggtgctggtggtactggtggtggtggaggtggtaaggttggaggaacttctgaaagctctgctgctattcacgctaccgctaagtggtctaccgctcagcttaagaaaaccctggctgagaaggctgctagagagagagaaactgctgctgcaatggctgctgctaaggctaagagagatgctcttacccagcacctgaaggatatcgtgaacgatgtgcttaggcacaacgcttctaggaccccttctgctactgatcttgctcacgctaacaacatggctatgcaggctgaagctcagagacttggtagagctaaggctgaggaaaaggctagaaaagaggctgaggctgctgagcttgctttccaagaagctgaaagacagagggaagaggctgttagacagcttgctgaaactgagaggcagcttaagcaagctgaggaagagaagaggcttgctgctctttctgatgaggctagggctgttgagaacgctaggaagaatctggataccgcaaagtccgagctggctaatgtggattctgatatcgagaggcagaggtcccagctgtcatctcttgatgctgatgtgaagaaggctgaagagaacctgaggctgaccatgaggattaagggtaggatcggtaggaagatgcaggctaagtcacaggctatcgtggatgataagaaaaggatctactccgatgctgagaacgtgctgaataccatgaccgtgaataggaacctgaaggctcagcaggttaccgatgcagagaatgagcttaaggtggcaatcgataacctgaacagcagccagatgaagaacgctgtggatgctaccgtgtctttctaccagactctgaccgagaagtacggtgagaagtacagccttatcgctcaagagctggcagagaagtccaagggtaagaaaatcggaaatgtggatgaggctctggctgcattcgagaagtataaggatgtgctggataagaagttcagcaaggctgatagggatgctattgtgaacgctctgaagtccttcaactacgatgattgggctaagcacctggatcagttcgctaagtacctgaagatcaccggtcacgtgagcttcggttacgatgttgtgtctgatgtgctgaaggctagcgagactggtgattggaagcctctgttcattacccttgagcagaaggtgttggatactggtatgagctacctggtggtgctgatgttctctcttattgctggaaccaccctgggaatcttcggtgtggctattattaccgctatcctgtgcagcttcgtggataagtacatcctgaacgcactgaacgatgctctgggaatctaa

SEQ ID NO: 19 - DNA, 1584 bp, Artificial Sequence
  codon-optimized coding sequence for expressing ScolE1b
atgagcgataacaccattgcttactacgaggatggtgtgccttacagcgctgatggtcaagtggtgattgtgatcgatggtaagatgcctgtggataccggtgctggtggtactggtggtggtggaggtggtaaggttggaggaacttctgaaagctctgctgctattcacgctaccgctaagtggtctaaggctcagcttcagaagtccctggaagagaaggctgctagagagagagaaactgctgctgcaatggctgctgctaaggctaagagagatgctcttacccagcacctgaaggatatcgtgaacgatgtgctgaggtacaacgcttctaggactccttctgctaccgatcttgctcacgctaacaacatggctatgcaggctgaagctcagagacttggtagagctaaggctgaggaaaaggctagaaaagaggctgaggctgctgagaagtctcttcaagaagctgagagacagagggaagaagctgctaggcaaagagctgaagcagagaggcaacttaagcaggcagaggctgaagagaagaggttggctgctctttctgaagaggctagggcagttgagatcacccagaagaatcttgctgctgctcagagcgagctgtccaagatggatggtgagatcaagagccttaacgtgaggctgtctacctctatccatgctagggatgctgagatgaacagcctgtctggtaagaggaacgagctggctcaagagagcgctaagtacaaagaactggatgagctggtgaagaagcttgagcctagggctaatgatcctctgcagaacaggcctttcttcgatgctacatctagaagggcaagggctggtgatactttggctgagaagcagaaagaggtgaccgcttctgagactaggatcaacgagcttaacaccgagatcaaccaggtgaggggtgctatttcacaggcaaacaacaataggaacctgaaggtgcagcaggttaccgagactgagaacgctcttaaggtggcaatcgataacctgaacagcagccagatgaagaacgctgtggatgctaccgtgtctttctaccagaccctgactgctaagtacggtgagaagtacagcctgatcgctcaagaacttgctgagcagtccaagggtaagaaaatcagcaatgtggatgaggctctggctgcattcgagaagtataaggatgtgctggataagaagttcagcaaggctgatagggatgcaattgtgaacgctctgaagtccgtggattacgctgattgggctaagcacctggatcagttcagcagatacctgaagatcagcggtagggtgtcaaccggttacgatatctacagcgatatcagaaagggtatggataccaacgattggaggcctctgttcctgacccttgagaagcttgctgttgatgctggtgtgggttacatcgtggctcttggtttctctgtgatcgcttctaccgctcttggtatttggggtgtggctattatcaccggtgtgatctgcagcttcgttgataagaaggatttggagaagctgaacgaggcactgggaatctaa

SEQ ID NO: 20 - DNA, 891 bp, Artificial Sequence
  codon-optimized coding sequence for expressing salmocin Spst
atgttcatcaagagcggtggtaacctgaccatcaggacttttggtggtcttggtgtgggtggtgatttcgatagcgatacttggagaagaaggtccaccgattcttgggtgccatacagcgagtacattgctatcgagtgcatcgtggctcctaaccagctttaccagcttcttactgatgtggctcaggtggaaactgtggctgctcaacttgctcaggttggataccagtatcttcagggtaggcttaggctggtgagagaggatggttcttgcaccgatttcagcggtaaggctatgctggataacctgctgaacaagagcaaggatattctggatctggatttcctgcacgtgagcgagggttataggtctgaagcttattggcctggtcagtcctctggtatcaccattggttacggtgtggatatcggtcaccagtctgaagagggacttcataagtggggtgtgcctcagagcatcatcgataagatcaaggattacttcggtattaccggtgaggctgctaacacccttcttaagggtctgaaggataagaccctgggactgagcgatagagagatcaagcagttctccgatatcgtgaagaagcaggctaccgctgatatcatcaacaagtacaacgctgctaccaagggtatcacctttgataagatcccttacaacaccaggaccgctatcatcgatctgttctaccagtacagcgctcctaagggtgctcctaagtcttggggtttcattatcaacaacgattggaacggtttctacaacgagctgatgaacttcggtgataagcacaccaccagaagagagagggaagctgctctggttctgtctgatattgtgaacaaccagtacatctacaagtaa

SEQ ID NO: 21 - DNA, 258 bp, Artificial Sequence
  codon-optimized coding sequence for expressing SImmE2
atggaactgaagaagtccatcagcgattacaccgaggctgagttcaagaagatcatcgaggctatcatcaactgcgagggtgatgagaaaacccaggatgataaccttgagttcttcatcagggtgaccgagtacccttctggtagcgatcttatctactaccctgagggtgataacgatggtagcaccgaggcaattatcaaagaaatcaaggaatggagggctgctaacggtaagcctggttttaagcaagcttaa

SEQ ID NO: 22 - DNA, 264 bp, Artificial Sequence
  codon-optimized coding sequence for expressing SImmE7
atggaactgaagaacagcatcagcgattacaccgaggctgagttcatcgagttcatgaaagaaatcgataaggaaaacgtggcagagactgatgataagctggatctgctgctgaaccacttcgagcaggttacagaacaccctgatggaaccgatctgatctactacgctgcttccgatgctgagtctacccctgaggctatcaccaagaaaatcaaagaatggagggctgctaacggtaagcctggttttaagcaaggttaa

SEQ ID NO: 23 - DNA, 15014 bp, Artificial Sequence
  nucleotide sequence of binary TMV-based vector used for salmocin ScolE1a expression
catggctgataacaccattgcttactacgaggatggtgtgcctcacagcgctgatggtaaggtggtgattgtgatcgatggtaagatgcctgtggataccggtgctggtggtactggtggtggtggaggtggtaaggttggaggaacttctgaaagctctgctgctattcacgctaccgctaagtggtctaccgctcagcttaagaaaaccctggctgagaaggctgctagagagagagaaactgctgctgcaatggctgctgctaaggctaagagagatgctcttacccagcacctgaaggatatcgtgaacgatgtgcttaggcacaacgcttctaggaccccttctgctactgatcttgctcacgctaacaacatggctatgcaggctgaagctcagagacttggtagagctaaggctgaggaaaaggctagaaaagaggctgaggctgctgagcttgctttccaagaagctgaaagacagagggaagaggctgttagacagcttgctgaaactgagaggcagcttaagcaagctgaggaagagaagaggcttgctgctctttctgatgaggctagggctgttgagaacgctaggaagaatctggataccgcaaagtccgagctggctaatgtggattctgatatcgagaggcagaggtcccagctgtcatctcttgatgctgatgtgaagaaggctgaagagaacctgaggctgaccatgaggattaagggtaggatcggtaggaagatgcaggctaagtcacaggctatcgtggatgataagaaaaggatctactccgatgctgagaacgtgctgaataccatgaccgtgaataggaacctgaaggctcagcaggttaccgatgcagagaatgagcttaaggtggcaatcgataacctgaacagcagccagatgaagaacgctgtggatgctaccgtgtctttctaccagactctgaccgagaagtacggtgagaagtacagccttatcgctcaagagctggcagagaagtccaagggtaagaaaatcggaaatgtggatgaggctctggctgcattcgagaagtataaggatgtgctggataagaagttcagcaaggctgatagggatgctattgtgaacgctctgaagtccttcaactacgatgattgggctaagcacctggatcagttcgctaagtacctgaagatcaccggtcacgtgagcttcggttacgatgttgtgtctgatgtgctgaaggctagcgagactggtgattggaagcctctgttcattacccttgagcagaaggtgttggatactggtatgagctacctggtggtgctgatgttctctcttattgctggaaccaccctgggaatcttcggtgtggctattattaccgctatcctgtgcagcttcgtggataagtacatcctgaacgcactgaacgatgctctgggaatctaagcttactagagcgtggtgcgcacgatagcgcatagtgtttttctctccacttgaatcgaagagatagacttacggtgtaaatccgtaggggtggcgtaaaccaaattacgcaatgttttgggttccatttaaatcgaaaccccttatttcctggatcacctgttaacgcacgtttgacgtgtattacagtgggaataagtaaaagtgagaggttcgaatcctccctaaccccgggtaggggcccagcggccgctctagctagagtcaagcagatcgttcaaacatttggcaataaagtttcttaagattgaatcctgttgccggtcttgcgatgattatcatataatttctgttgaattacgttaagcatgtaataattaacatgtaatgcatgacgttatttatgagatgggtttttatgattagagtcccgcaattatacatttaatacgcgatagaaaacaaaatatagcgcgcaaactaggataaattatcgcgcgcggtgtcatctatgttactagatcgacctgcatccaccccagtacattaaaaacgtccgcaatgtgttattaagttgtctaagcgtcaatttgtttacaccacaatatatcctgccaccagccagccaacagctccccgaccggcagctcggcacaaaatcaccactcgatacaggcagcccatcagtcagatcaggatctcctttgcgacgctcaccgggctggttgccctcgccgctgggctggcggccgtctatggccctgcaaacgcgccagaaacgccgtcgaagccgtgtgcgagacaccgcggccgccggcgttgtggatacctcgcggaaaacttggccctcactgacagatgaggggcggacgttgacacttgaggggccgactcacccggcgcggcgttgacagatgaggggcaggctcgatttcggccggcgacgtggagctggccagcctcgcaaatcggcgaaaacgcctgattttacgcgagtttcccacagatgatgtggacaagcctggggataagtgccctgcggtattgacacttgaggggcgcgactactgacagatgaggggcgcgatccttgacacttgaggggcagagtgctgacagatgaggggcgcacctattgacatttgaggggctgtccacaggcagaaaatccagcatttgcaagggtttccgcccgtttttcggccaccgctaacctgtcttttaacctgcttttaaaccaatatttataaaccttgtttttaaccagggctgcgccctgtgcgcgtgaccgcgcacgccgaaggggggtgcccccccttctcgaaccctcccggcccgctaacgcgggcctcccatccccccaggggctgcgcccctcggccgcgaacggcctcaccccaaaaatggcagcgctggccaattcgtgcgcggaacccctatttgtttatttttctaaatacattcaaatatgtatccgctcatgagacaataaccctgataaatgcttcaataatattgaaaaaggaagagtatggctaaaatgagaatatcaccggaattgaaaaaactgatcgaaaaataccgctgcgtaaaagatacggaaggaatgtctcctgctaaggtatataagctggtgggagaaaatgaaaacctatatttaaaaatgacggacagccggtataaagggaccacctatgatgtggaacgggaaaaggacatgatgctatggctggaaggaaagctgcctgttccaaaggtcctgcactttgaacggcatgatggctggagcaatctgctcatgagtgaggccgatggcgtcctttgctcggaagagtatgaagatgaacaaagccctgaaaagattatcgagctgtatgcggagtgcatcaggctctttcactccatcgacatatcggattgtccctatacgaatagcttagacagccgcttagccgaattggattacttactgaataacgatctggccgatgtggattgcgaaaactgggaagaagacactccatttaaagatccgcgcgagctgtatgattttttaaagacggaaaagcccgaagaggaacttgtcttttcccacggcgacctgggagacagcaacatctttgtgaaagatggcaaagtaagtggctttattgatcttgggagaagcggcagggcggacaagtggtatgacattgccttctgcgtccggtcgatcagggaggatatcggggaagaacagtatgtcgagctattttttgacttactggggatcaagcctgattgggagaaaataaaatattatattttactggatgaattgttttagctgtcagaccaagtttactcatatatactttagattgatttaaaacttcatttttaatttaaaaggatctaggtgaagatcctttttgataatctcatgaccaaaatcccttaacgtgagttttcgttccactgagcgtcagaccccgtagaaaagatcaaaggatcttcttgagatcctttttttctgcgcgtaatctgctgcttgcaaacaaaaaaaccaccgctaccagcggtggtttgtttgccggatcaagagctaccaactctttttccgaaggtaactggcttcagcagagcgcagataccaaatactgtccttctagtgtagccgtagttaggccaccacttcaagaactctgtagcaccgcctacatacctcgctctgctaatcctgttaccagtggctgctgccagtggcgataagtcgtgtcttaccgggttggactcaagacgatagttaccggataaggcgcagcggtcgggctgaacggggggttcgtgcacacagcccagcttggagcgaacgacctacaccgaactgagatacctacagcgtgagctatgagaaagcgccacgcttcccgaagggagaaaggcggacaggtatccggtaagcggcagggtcggaacaggagagcgcacgagggagcttccagggggaaacgcctggtatctttatagtcctgtcgggtttcgccacctctgacttgagcgtcgatttttgtgatgctcgtcaggggggcggagcctatggaaaaacgccagcaacgcggcctttttacggttcctggcagatcctagatgtggcgcaacgatgccggcgacaagcaggagcgcaccgacttcttccgcatcaagtgttttggctctcaggccgaggcccacggcaagtatttgggcaaggggtcgctggtattcgtgcagggcaagattcggaataccaagtacgagaaggacggccagacggtctacgggaccgacttcattgccgataaggtggattatctggacaccaaggcaccaggcgggtcaaatcaggaataagggcacattgccccggcgtgagtcggggcaatcccgcaaggagggtgaatgaatcggacgtttgaccggaaggcatacaggcaagaactgatcgacgcggggttttccgccgaggatgccgaaaccatcgcaagccgcaccgtcatgcgtgcgccccgcgaaaccttccagtccgtcggctcgatggtccagcaagctacggccaagatcgagcgcgacagcgtgcaactggctccccctgccctgcccgcgccatcggccgccgtggagcgttcgcgtcgtctcgaacaggaggcggcaggtttggcgaagtcgatgaccatcgacacgcgaggaactatgacgaccaagaagcgaaaaaccgccggcgaggacctggcaaaacaggtcagcgaggccaagcaggccgcgttgctgaaacacacgaagcagcagatcaaggaaatgcagctttccttgttcgatattgcgccgtggccggacacgatgcgagcgatgccaaacgacacggcccgctctgccctgttcaccacgcgcaacaagaaaatcccgcgcgaggcgctgcaaaacaaggtcattttccacgtcaacaaggacgtgaagatcacctacaccggcgtcgagctgcgggccgacgatgacgaactggtgtggcagcaggtgttggagtacgcgaagcgcacccctatcggcgagccgatcaccttcacgttctacgagctttgccaggacctgggctggtcgatcaatggccggtattacacgaaggccgaggaatgcctgtcgcgcctacaggcgacggcgatgggcttcacgtccgaccgcgttgggcacctggaatcggtgtcgctgctgcaccgcttccgcgtcctggaccgtggcaagaaaacgtcccgttgccaggtcctgatcgacgaggaaatcgtcgtgctgtttgctggcgaccactacacgaaattcatatgggagaagtaccgcaagctgtcgccgacggcccgacggatgttcgactatttcagctcgcaccgggagccgtacccgctcaagctggaaaccttccgcctcatgtgcggatcggattccacccgcgtgaagaagtggcgcgagcaggtcggcgaagcctgcgaagagttgcgaggcagcggcctggtggaacacgcctgggtcaatgatgacctggtgcattgcaaacgctagggccttgtggggtcagttccggctgggggttcagcagccagcgcctgatctggggaaccctgtggttggcacatacaaatggacgaacggataaaccttttcacgcccttttaaatatccgattattctaataaacgctcttttctcttaggtttacccgccaatatatcctgtcaaacactgatagtttaaactgaaggcgggaaacgacaatctgatctaagctagcttggaattggtaccacgcgtttcgacaaaatttagaacgaacttaattatgatctcaaatacattgatacatatctcatctagatctaggttatcattatgtaagaaagttttgacgaatatggcacgacaaaatggctagactcgatgtaattggtatctcaactcaacattatacttataccaaacattagttagacaaaatttaaacaactattttttatgtatgcaagagtcagcatatgtataattgattcagaatcgttttgacgagttcggatgtagtagtagccattatttaatgtacatactaatcgtgaatagtgaatatgatgaaacattgtatcttattgtataaatatccataaacacatcatgaaagacactttctttcacggtctgaattaattatgatacaattctaatagaaaacgaattaaattacgttgaattgtatgaaatctaattgaacaagccaaccacgacgacgactaacgttgcctggattgactcggtttaagttaaccactaaaaaaacggagctgtcatgtaacacgcggatcgagcaggtcacagtcatgaagccatcaaagcaaaagaactaatccaagggctgagatgattaattagtttaaaaattagttaacacgagggaaaaggctgtctgacagccaggtcacgttatctttacctgtggtcgaaatgattcgtgtctgtcgattttaattatttttttgaaaggccgaaaataaagttgtaagagataaacccgcctatataaattcatatattttcctctccgctttgaagttttagttttattgcaacaacaacaacaaattacaataacaacaaacaaaatacaaacaacaacaacatggcacaatttcaacaaacaattgacatgcaaactctccaagccgctgcgggacgcaacagcttggtgaatgatttggcatctcgtcgcgtttacgataatgcagtcgaggagctgaatgctcgttccagacgtcccaaggtaataggaactttctggatctactttatttgctggatctcgatcttgttttctcaatttccttgagatctggaattcgtttaatttggatctgtgaacctccactaaatcttttggttttactagaatcgatctaagttgaccgatcagttagctcgattatagctaccagaatttggcttgaccttgatggagagatccatgttcatgttacctgggaaatgatttgtatatgtgaattgaaatctgaactgttgaagttagattgaatctgaacactgtcaatgttagattgaatctgaacactgtttaaggttagatgaagtttgtgtatagattcttcgaaactttaggatttgtagtgtcgtacgttgaacagaaagctatttctgattcaatcagggtttatttgactgtattgaactctttttgtgtgtttgcaggtccacttctccaaggcagtgtctacggaacagaccctgattgcaacaaacgcatatccggagttcgagatttcctttactcatacgcaatccgctgtgcactccttggccggaggccttcggtcacttgagttggagtatctcatgatgcaagttccgttcggttctctgacgtacgacatcggcggtaacttttccgcgcaccttttcaaagggcgcgattacgttcactgctgcatgcctaatctggatgtacgtgacattgctcgccatgaaggacacaaggaagctatttacagttatgtgaatcgtttgaaaaggcagcagcgtcctgtgcctgaataccagagggcagctttcaacaactacgctgagaacccgcacttcgtccattgcgacaaacctttccaacagtgtgaattgacgacagcgtatggcactgacacctacgctgtagctctccatagcatttatgatatccctgttgaggagttcggttctgcgctactcaggaagaatgtgaaaacttgtttcgcggcctttcatttccatgagaatatgcttctagattgtgatacagtcacactcgatgagattggagctacgttccagaaatcaggtaacattccttagttacctttcttttctttttccatcataagtttatagattgtacatgctttgagatttttctttgcaaacaatctcaggtgataacctgagcttcttcttccataatgagagcactctcaattacacccacagcttcagcaacatcatcaagtacgtgtgcaagacgttcttccctgctagtcaacgcttcgtgtaccacaaggagttcctggtcactagagtcaacacttggtactgcaagttcacgagagtggatacgttcactctgttccgtggtgtgtaccacaacaatgtggattgcgaagagttttacaaggctatggacgatgcgtggcactacaaaaagacgttagcaatgcttaatgccgagaggaccatcttcaaggataacgctgcgttaaacttctggttcccgaaggtgctcttgaaattggaagtcttcttttgttgtctaaacctatcaatttctttgcggaaatttatttgaagctgtagagttaaaattgagtcttttaaacttttgtaggtgagagacatggttatcgtccctctctttgacgcttctatcacaactggtaggatgtctaggagagaggttatggtgaacaaggacttcgtctacacggtcctaaatcacatcaagacctatcaagctaaggcactgacgtacgcaaacgtgctgagcttcgtggagtctattaggtctagagtgataattaacggtgtcactgccaggtaagttgttacttatgattgttttcctctctgctacatgtattttgttgttcatttctgtaagatataagaattgagttttcctctgatgatattattaggtctgaatgggacacagacaaggcaattctaggtccattagcaatgacattcttcctgatcacgaagctgggtcatgtgcaagatgaaataatcctgaaaaagttccagaagttcgacagaaccaccaatgagctgatttggacaagtctctgcgatgccctgatgggggttattccctcggtcaaggagacgcttgtgcgcggtggttttgtgaaagtagcagaacaagccttagagatcaaggttagtatcatatgaagaaatacctagtttcagttgatgaatgctattttctgacctcagttgttctcttttgagaattatttcttttctaatttgcctgatttttctattaattcattaggttcccgagctatactgtaccttcgccgaccgattggtactacagtacaagaaggcggaggagttccaatcgtgtgatctttccaaacctctagaagagtcagagaagtactacaacgcattatccgagctatcagtgcttgagaatctcgactcttttgacttagaggcgtttaagactttatgtcagcagaagaatgtggacccggatatggcagcaaaggtaaatcctggtccacacttttacgataaaaacacaagattttaaactatgaactgatcaataatcattcctaaaagaccacacttttgttttgtttctaaagtaatttttactgttataacaggtggtcgtagcaatcatgaagtcagaattgacgttgcctttcaagaaacctacagaagaggaaatctcggagtcgctaaaaccaggagaggggtcgtgtgcagagcataaggaagtgttgagcttacaaaatgatgctccgttcccgtgtgtgaaaaatctagttgaaggttccgtgccggcgtatggaatgtgtcctaagggtggtggtttcgacaaattggatgtggacattgctgatttccatctcaagagtgtagatgcagttaaaaagggaactatgatgtctgcggtgtacacagggtctatcaaagttcaacaaatgaagaactacatagattacttaagtgcgtcgctggcagctacagtctcaaacctctgcaaggtaagaggtcaaaaggtttccgcaatgatccctctttttttgtttctctagtttcaagaatttgggtatatgactaacttctgagtgttccttgatgcatatttgtgatgagacaaatgtttgttctatgttttaggtgcttagagatgttcacggcgttgacccagagtcacaggagaaatctggagtgtgggatgttaggagaggacgttggttacttaaacctaatgcgaaaagtcacgcgtggggtgtggcagaagacgccaaccacaagttggttattgtgttactcaactgggatgacggaaagccggtttgtgatgagacatggttcagggtggcggtgtcaagcgattccttgatatattcggatatgggaaaacttaagacgctcacgtcttgcagtccaaatggtgagccaccggagcctaacgccaaagtaattttggtcgatggtgttcccggttgtggaaaaacgaaggagattatcgaaaaggtaagttctgcatttggttatgctccttgcattttaggtgttcgtcgctcttccatttccatgaatagctaagattttttttctctgcattcattcttcttgcctcagttctaactgtttgtggtatttttgttttaattattgctacaggtaaacttctctgaagacttgattttagtccctgggaaggaagcttctaagatgatcatccggagggccaaccaagctggtgtgataagagcggataaggacaatgttagaacggtggattccttcttgatgcatccttctagaagggtgtttaagaggttgtttatcgatgaaggactaatgctgcatacaggttgtgtaaatttcctactgctgctatctcaatgtgacgtcgcatatgtgtatggggacacaaagcaaattccgttcatttgcagagtcgcgaactttccgtatccagcgcattttgcaaaactcgtcgctgatgagaaggaagtcagaagagttacgctcaggtaaagcaactgtgttttaatcaatttcttgtcaggatatatggattataacttaatttttgagaaatctgtagtatttggcgtgaaatgagtttgctttttggtttctcccgtgttataggtgcccggctgatgttacgtatttccttaacaagaagtatgacggggcggtgatgtgtaccagcgcggtagagagatccgtgaaggcagaagtggtgagaggaaagggtgcattgaacccaataaccttaccgttggagggtaaaattttgaccttcacacaagctgacaagttcgagttactggagaagggttacaaggtaaagtttccaactttcctttaccatatcaaactaaagttcgaaactttttatttgatcaacttcaaggccacccgatctttctattcctgattaatttgtgatgaatccatattgacttttgatggttacgcaggatgtgaacactgtgcacgaggtgcaaggggagacgtacgagaagactgctattgtgcgcttgacatcaactccgttagagatcatatcgagtgcgtcacctcatgttttggtggcgctgacaagacacacaacgtgttgtaaatattacaccgttgtgttggacccgatggtgaatgtgatttcagaaatggagaagttgtccaatttccttcttgacatgtatagagttgaagcaggtctgtctttcctatttcatatgtttaatcctaggaatttgatcaattgattgtatgtatgtcgatcccaagactttcttgttcacttatatcttaactctctctttgctgtttcttgcaggtgtccaatagcaattacaaatcgatgcagtattcaggggacagaacttgtttgttcagacgcccaagtcaggagattggcgagatatgcaattttactatgacgctcttcttcccggaaacagtactattctcaatgaatttgatgctgttacgatgaatttgagggatatttccttaaacgtcaaagattgcagaatcgacttctccaaatccgtgcaacttcctaaagaacaacctattttcctcaagcctaaaataagaactgcggcagaaatgccgagaactgcaggtaaaatattggatgccagacgatattctttcttttgatttgtaactttttcctgtcaaggtcgataaattttattttttttggtaaaaggtcgataatttttttttggagccattatgtaattttcctaattaactgaaccaaaattatacaaaccaggtttgctggaaaatttggttgcaatgatcaaaagaaacatgaatgcgccggatttgacagggacaattgacattgaggatactgcatctctggtggttgaaaagttttgggattcgtatgttgacaaggaatttagtggaacgaacgaaatgaccatgacaagggagagcttctccaggtaaggacttctcatgaatattagtggcagattagtgttgttaaagtctttggttagataatcgatgcctcctaattgtccatgttttactggttttctacaattaaaggtggctttcgaaacaagagtcatctacagttggtcagttagcggactttaactttgtggatttgccggcagtagatgagtacaagcatatgatcaagagtcaaccaaagcaaaagttagacttgagtattcaagacgaatatcctgcattgcagacgatagtctaccattcgaaaaagatcaatgcgattttcggtccaatgttttcagaacttacgaggatgttactcgaaaggattgactcttcgaagtttctgttctacaccagaaagacacctgcacaaatagaggacttcttttctgacctagactcaacccaggcgatggaaattctggaactcgacatttcgaagtacgataagtcacaaaacgagttccattgtgctgtagagtacaagatctgggaaaagttaggaattgatgagtggctagctgaggtctggaaacaaggtgagttcctaagttccatttttttgtaatccttcaatgttattttaacttttcagatcaacatcaaaattaggttcaattttcatcaaccaaataatatttttcatgtatatataggtcacagaaaaacgaccttgaaagattatacggccggaatcaaaacatgtctttggtatcaaaggaaaagtggtgatgtgacaacctttattggtaataccatcatcattgccgcatgtttgagctcaatgatccccatggacaaagtgataaaggcagctttttgtggagacgatagcctgatttacattcctaaaggtttagacttgcctgatattcaggcgggcgcgaacctcatgtggaacttcgaggccaaactcttcaggaagaagtatggttacttctgtggtcgttatgttattcaccatgatagaggagccattgtgtattacgatccgcttaaactaatatctaagttaggttgtaaacatattagagatgttgttcacttagaagagttacgcgagtctttgtgtgatgtagctagtaacttaaataattgtgcgtatttttcacagttagatgaggccgttgccgaggttcataagaccgcggtaggcggttcgtttgctttttgtagtataattaagtatttgtcagataagagattgtttagagatttgttctttgtttgataatgtcgatagtctcgtacgaacctaaggtgagtgatttcctcaatctttcgaagaaggaagagatcttgccgaaggctctaacgaggttaaaaaccgtgtctattagtactaaagatattatatctgtcaaggagtcggagactttgtgtgatatagatttgttaatcaatgtgccattagataagtatagatatgtgggtatcctaggagccgtttttaccggagagtggctagtgccagacttcgttaaaggtggagtgacgataagtgtgatagataagcgtctggtgaactcaaaggagtgcgtgattggtacgtacagagccgcagccaagagtaagaggttccagttcaaattggttccaaattactttgtgtccaccgtggacgcaaagaggaagccgtggcaggtaaggatttttatgatatagtatgcttatgtattttgtactgaaagcatatcctgcttcattgggatattactgaaagcatttaactacatgtaaactcacttgatgatcaataaacttgattttgcaggttcatgttcgtatacaagacttgaagattgaggcgggttggcagccgttagctctggaagtagtttcagttgctatggtcaccaataacgttgtcatgaagggtttgagggaaaaggtcgtcgcaataaatgatccggacgtcgaaggtttcgaaggtaagccatcttcctgcttatttttataatgaacatagaaataggaagttgtgcagagaaactaattaacctgactcaaaatctaccctcataattgttgtttgatattggtcttgtattttgcaggtgtggttgacgaattcgtcgattcggttgcagcatttaaagcggttgacaactttaaaagaaggaaaaagaaggttgaagaaaagggtgtagtaagtaagtataagtacagaccggagaagtacgccggtcctgattcgtttaatttgaaagaagaaaacgtcttacaacattacaaacccgaatcagtaccagtatttcgataagaaacaagaaac

SEQ ID NO: 24 - DNA, 11586 bp, Artificial Sequence
  nucleotide sequence of binary PVX-based vector used for salmocin ImmScolE2 expression
gatcggtcgtatcactggaacaacaaccgctgaggctgttgtcactctaccaccaccataactacgtctacataaccgacgcctaccccagtttcatagtattttctggtttgattgtatgaataatataaataaaaaaaaaaaaaaaaaaaaaaaactagtgagctcttctgtcagcgggcccactgcatccaccccagtacattaaaaacgtccgcaatgtgttattaagttgtctaagcgtcaatttgtttacaccacaatatatcctgccaccagccagccaacagctccccgaccggcagctcggcacaaaatcaccactcgatacaggcagcccatcagtcagatcaggatctcctttgcgacgctcaccgggctggttgccctcgccgctgggctggcggccgtctatggccctgcaaacgcgccagaaacgccgtcgaagccgtgtgcgagacaccgcggccgccggcgttgtggatacctcgcggaaaacttggccctcactgacagatgaggggcggacgttgacacttgaggggccgactcacccggcgcggcgttgacagatgaggggcaggctcgatttcggccggcgacgtggagctggccagcctcgcaaatcggcgaaaacgcctgattttacgcgagtttcccacagatgatgtggacaagcctggggataagtgccctgcggtattgacacttgaggggcgcgactactgacagatgaggggcgcgatccttgacacttgaggggcagagtgctgacagatgaggggcgcacctattgacatttgaggggctgtccacaggcagaaaatccagcatttgcaagggtttccgcccgtttttcggccaccgctaacctgtcttttaacctgcttttaaaccaatatttataaaccttgtttttaaccagggctgcgccctgtgcgcgtgaccgcgcacgccgaaggggggtgcccccccttctcgaaccctcccggcccgctaacgcgggcctcccatccccccaggggctgcgcccctcggccgcgaacggcctcaccccaaaaatggcagcgctggccaattcgtgcgcggaacccctatttgtttatttttctaaatacattcaaatatgtatccgctcatgagacaataaccctgataaatgcttcaataatattgaaaaaggaagagtatggctaaaatgagaatatcaccggaattgaaaaaactgatcgaaaaataccgctgcgtaaaagatacggaaggaatgtctcctgctaaggtatataagctggtgggagaaaatgaaaacctatatttaaaaatgacggacagccggtataaagggaccacctatgatgtggaacgggaaaaggacatgatgctatggctggaaggaaagctgcctgttccaaaggtcctgcactttgaacggcatgatggctggagcaatctgctcatgagtgaggccgatggcgtcctttgctcggaagagtatgaagatgaacaaagccctgaaaagattatcgagctgtatgcggagtgcatcaggctctttcactccatcgacatatcggattgtccctatacgaatagcttagacagccgcttagccgaattggattacttactgaataacgatctggccgatgtggattgcgaaaactgggaagaagacactccatttaaagatccgcgcgagctgtatgattttttaaagacggaaaagcccgaagaggaacttgtcttttcccacggcgacctgggagacagcaacatctttgtgaaagatggcaaagtaagtggctttattgatcttgggagaagcggcagggcggacaagtggtatgacattgccttctgcgtccggtcgatcagggaggatatcggggaagaacagtatgtcgagctattttttgacttactggggatcaagcctgattgggagaaaataaaatattatattttactggatgaattgttttagctgtcagaccaagtttactcatatatactttagattgatttaaaacttcatttttaatttaaaaggatctaggtgaagatcctttttgataatctcatgaccaaaatcccttaacgtgagttttcgttccactgagcgtcagaccccgtagaaaagatcaaaggatcttcttgagatcctttttttctgcgcgtaatctgctgcttgcaaacaaaaaaaccaccgctaccagcggtggtttgtttgccggatcaagagctaccaactctttttccgaaggtaactggcttcagcagagcgcagataccaaatactgtccttctagtgtagccgtagttaggccaccacttcaagaactctgtagcaccgcctacatacctcgctctgctaatcctgttaccagtggctgctgccagtggcgataagtcgtgtcttaccgggttggactcaagacgatagttaccggataaggcgcagcggtcgggctgaacggggggttcgtgcacacagcccagcttggagcgaacgacctacaccgaactgagatacctacagcgtgagctatgagaaagcgccacgcttcccgaagggagaaaggcggacaggtatccggtaagcggcagggtcggaacaggagagcgcacgagggagcttccagggggaaacgcctggtatctttatagtcctgtcgggtttcgccacctctgacttgagcgtcgatttttgtgatgctcgtcaggggggcggagcctatggaaaaacgccagcaacgcggcctttttacggttcctggcagatcctagatgtggcgcaacgatgccggcgacaagcaggagcgcaccgacttcttccgcatcaagtgttttggctctcaggccgaggcccacggcaagtatttgggcaaggggtcgctggtattcgtgcagggcaagattcggaataccaagtacgagaaggacggccagacggtctacgggaccgacttcattgccgataaggtggattatctggacaccaaggcaccaggcgggtcaaatcaggaataagggcacattgccccggcgtgagtcggggcaatcccgcaaggagggtgaatgaatcggacgtttgaccggaaggcatacaggcaagaactgatcgacgcggggttttccgccgaggatgccgaaaccatcgcaagccgcaccgtcatgcgtgcgccccgcgaaaccttccagtccgtcggctcgatggtccagcaagctacggccaagatcgagcgcgacagcgtgcaactggctccccctgccctgcccgcgccatcggccgccgtggagcgttcgcgtcgtctcgaacaggaggcggcaggtttggcgaagtcgatgaccatcgacacgcgaggaactatgacgaccaagaagcgaaaaaccgccggcgaggacctggcaaaacaggtcagcgaggccaagcaggccgcgttgctgaaacacacgaagcagcagatcaaggaaatgcagctttccttgttcgatattgcgccgtggccggacacgatgcgagcgatgccaaacgacacggcccgctctgccctgttcaccacgcgcaacaagaaaatcccgcgcgaggcgctgcaaaacaaggtcattttccacgtcaacaaggacgtgaagatcacctacaccggcgtcgagctgcgggccgacgatgacgaactggtgtggcagcaggtgttggagtacgcgaagcgcacccctatcggcgagccgatcaccttcacgttctacgagctttgccaggacctgggctggtcgatcaatggccggtattacacgaaggccgaggaatgcctgtcgcgcctacaggcgacggcgatgggcttcacgtccgaccgcgttgggcacctggaatcggtgtcgctgctgcaccgcttccgcgtcctggaccgtggcaagaaaacgtcccgttgccaggtcctgatcgacgaggaaatcgtcgtgctgtttgctggcgaccactacacgaaattcatatgggagaagtaccgcaagctgtcgccgacggcccgacggatgttcgactatttcagctcgcaccgggagccgtacccgctcaagctggaaaccttccgcctcatgtgcggatcggattccacccgcgtgaagaagtggcgcgagcaggtcggcgaagcctgcgaagagttgcgaggcagcggcctggtggaacacgcctgggtcaatgatgacctggtgcattgcaaacgctagggccttgtggggtcagttccggctgggggttcagcagccagcgcctgatctggggaaccctgtggttggcacatacaaatggacgaacggataaaccttttcacgcccttttaaatatccgattattctaataaacgctcttttctcttaggtttacccgccaatatatcctgtcaaacactgatagtttaaactgaaggcgggaaacgacaatctgatctaagctaggcatgcctgcaggtcaacatggtggagcacgacacgcttgtctactccaaaaatatcaaagatacagtctcagaagaccaaagggcaattgagacttttcaacaaagggtaatatccggaaacctcctcggattccattgcccagctatctgtcactttattgtgaagatagtggaaaaggaaggtggctcctacaaatgccatcattgcgataaaggaaaggccatcgttgaagatgcctctgccgacagtggtcccaaagatggacccccacccacgaggagcatcgtggaaaaagaagacgttccaaccacgtcttcaaagcaagtggattgatgtgatatctccactgacgtaagggatgacgcacaatcccactatccttcgcaagacccttcctctatataaggaagttcatttcatttggagaggagaaaactaaaccatacaccaccaacacaaccaaacccaccacgcccaattgttacacacccgcttgaaaaagaaagtttaacaaatggccaaggtgcgcgaggtttaccaatcttttacagactccaccacaaaaactctcatccaagatgaggcttatagaaacattcgccccatcatggaaaaacacaaactagctaacccttacgctcaaacggttgaagcggctaatgatctagaggggttcggcatagccaccaatccctatagcattgaattgcatacacatgcagccgctaagaccatagagaataaacttctagaggtgcttggttccatcctaccacaagaacctgttacatttatgtttcttaaacccagaaagctaaactacatgagaagaaacccgcggatcaaggacattttccaaaatgttgccattgaaccaagagacgtagccaggtaccccaaggaaacaataattgacaaactcacagagatcacaacggaaacagcatacattagtgacactctgcacttcttggatccgagctacatagtggagacattccaaaactgcccaaaattgcaaacattgtatgcgaccttagttctccccgttgaggcagcctttaaaatggaaagcactcacccgaacatatacagcctcaaatacttcggagatggtttccagtatataccaggcaaccatggtggcggggcataccatcatgaattcgctcatctacaatggctcaaagtgggaaagatcaagtggagggaccccaaggatagctttctcggacatctcaattacacgactgagcaggttgagatgcacacagtgacagtacagttgcaggaatcgttcgcggcaaaccacttgtactgcatcaggagaggagacttgctcacaccggaggtgcgcactttcggccaacctgacaggtacgtgattccaccacagatcttcctcccaaaagttcacaactgcaagaagccgattctcaagaaaactatgatgcagctcttcttgtatgttaggacagtcaaggtcgcaaaaaattgtgacatttttgccaaagtcagacaattaattaaatcatctgacttggacaaatactctgctgtggaactggtttacttagtaagctacatggagttccttgccgatttacaagctaccacctgcttctcagacacactttctggtggcttgctaacaaagacccttgcaccggtgagggcttggatacaagagaaaaagatgcagctgtttggtcttgaggactacgcgaagttagtcaaagcagttgatttccacccggtggatttttctttcaaagtggaaacttgggacttcagattccaccccttgcaagcgtggaaagccttccgaccaagggaagtgtcggatgtagaggaaatggaaagtttgttctcagatggggacctgcttgattgcttcacaagaatgccagcttatgcggtaaacgcagaggaagatttagctgcaatcaggaaaacgcccgagatggatgtcggtcaagaagttaaagagcctgcaggagacagaaatcaatactcaaaccctgcagaaactttcctcaacaagctccacaggaaacacagtagggaggtgaaacaccaggccgcaaagaaagctaaacgcctagctgaaatccaggagtcaatgagagctgaaggtgatgccgaaccaaatgaaataagcgggacgatgggggcaatacccagcaacgccgaacttcctggcacgaatgatgccagacaagaactcacactcccaaccactaaacctgtccctgcaaggtgggaagatgcttcattcacagattctagtgtggaagaggagcaggttaaactccttggaaaagaaaccgttgaaacagcgacgcaacaagtcatcgaaggacttccttggaaacactggattcctcaattaaatgctgttggattcaaggcgctggaaattcagagggataggagtggaacaatgatcatgcccatcacagaaatggtgtccgggctggaaaaagaggacttccctgaaggaactccaaaagagttggcacgagaattgttcgctatgaacagaagccctgccaccatccctttggacctgcttagagccagagactacggcagtgatgtaaagaacaagagaattggtgccatcacaaagacacaggcaacgagttggggcgaatacttgacaggaaagatagaaagcttaactgagaggaaagttgcgacttgtgtcattcatggagctggaggttctggaaaaagtcatgccatccagaaggcattgagagaaattggcaagggctcggacatcactgtagtcctgccgaccaatgaactgcggctagattggagtaagaaagtgcctaacactgagccctatatgttcaagacctctgaaaaggcgttaattgggggaacaggcagcatagtcatctttgacgattactcaaaacttcctcccggttacatagaagccttagtctgtttctactctaaaatcaagctaatcattctaacaggagatagcagacaaagcgtctaccatgaaactgctgaggacgcctccatcaggcatttgggaccagcaacagagtacttctcaaaatactgccgatactatctcaatgccacacaccgcaacaagaaagatcttgcgaacatgcttggtgtctacagtgagagaacgggagtcaccgaaatcagcatgagcgccgagttcttagaaggaatcccaactttggtaccctcggatgagaagagaaagctgtacatgggcaccgggaggaatgacacgttcacatacgctggatgccaggggctaactaagccgaaggtacaaatagtgttggaccacaacacccaagtgtgtagcgcgaatgtgatgtacacggcactttctagagccaccgataggattcacttcgtgaacacaagtgcaaattcctctgccttctgggaaaagttggacagcaccccttacctcaagactttcctatcagtggtgagagaacaagcactcagggagtacgagccggcagaggcagagccaattcaagagcctgagccccagacacacatgtgtgtcgagaatgaggagtccgtgctagaagagtacaaagaggaactcttggaaaagtttgacagagagatccactctgaatcccatggtcattcaaactgtgtccaaactgaagacacaaccattcagttgttttcgcatcaacaagcaaaagatgagactctcctctgggcgactatagatgcgcggctcaagaccagcaatcaagaaacaaacttccgagaattcctgagcaagaaggacattggggacgttctgtttttaaactaccaaaaagctatgggtttacccaaagagcgtattcctttttcccaagaggtctgggaagcttgtgcccacgaagtacaaagcaagtacctcagcaagtcaaagtgcaacttgatcaatgggactgtgagacagagcccagacttcgatgaaaataagattatggtattcctcaagtcgcagtgggtcacaaaggtggaaaaactaggtctacccaagattaagccaggtcaaaccatagcagccttttaccagcagactgtgatgctttttggaactatggctaggtacatgcgatggttcagacaggctttccagccaaaagaagtcttcataaactgtgagacgacgccagatgacatgtctgcatgggccttgaacaactggaatttcagcagacctagcttggctaatgactacacagctttcgaccagtctcaggatggagccatgttgcaatttgaggtgctcaaagccaaacaccactgcataccagaggaaatcattcaggcatacatagatattaagactaatgcacagattttcctaggcacgttatcaattatgcgcctgactggtgaaggtcccacttttgatgcaaacactgagtgcaacatagcttacacccatacaaagtttgacatcccagccggaactgctcaagtttatgcaggagacgactccgcactggactgtgttccagaagtgaagcatagtttccacaggcttgaggacaaattactcctaaagtcaaagcctgtaatcacgcagcaaaagaagggcagttggcctgagttttgtggttggctgatcacaccaaaaggggtgatgaaagacccaattaagctccatgttagcttaaaattggctgaagctaagggtgaactcaagaaatgtcaagattcctatgaaattgatctgagttatgcctatgaccacaaggactctctgcatgacttgttcgatgagaaacagtgtcaggcacacacactcacttgcagaacactaatcaagtcagggagaggcactgtctcactttcccgcctcagaaactttctttaaccgttaagttaccttagagatttgaataagatgtcagcaccagctagtacaacacagcccatagggtcaactacctcaactaccacaaaaactgcaggcgcaactcctgccacagcttcaggcctgttcactatcccggatggggatttctttagtacagcccgtgccatagtagccagcaatgctgtcgcaacaaatgaggacctcagcaagattgaggctatttggaaggacatgaaggtgcccacagacactatggcacaggctgcttgggacttagtcagacactgtgctgatgtaggatcatccgctcaaacagaaatgatagatacaggtccctattccaacggcatcagcagagctagactggcagcagcaattaaagaggtgtgcacacttaggcaattttgcatgaagtatgccccagtggtatggaactggatgttaactaacaacagtccacctgctaactggcaagcacaaggtttcaagcctgagcacaaattcgctgcattcgacttcttcaatggagtcaccaacccagctgccatcatgcccaaagaggggctcatccggccaccgtctgaagctgaaatgaatgctgcccaaactgctgcctttgtgaagattacaaaggccagggcacaatccaacgactttgccagcctagatgcagctgtcactcgaggaaggatcaccggaacgaccacagcagaggcagtcgttactctgcctcctccataacagaaactttctttaaccgttaagttaccttagagatttgaataagatggatattctcatcagtagtttgaaaagtttaggttattctaggacttccaaatctttagattcaggacctttggtagtacatgcagtagccggagccggtaagtccacagccctaaggaagttgatcctcagacacccaacattcaccgtgcatacactcggtgtccctgacaaggtgagtatcagaactagaggcatacagaagccaggacctattcctgagggcaacttcgcaatcctcgatgagtatactttggacaacaccacaaggaactcataccaggcactttttgctgacccttatcaggcaccggagtttagcctagagccccacttctacttggaaacatcatttcgagttccgaggaaagtggcagatttgatagctggctgtggcttcgatttcgagacgaactcaccggaagaagggcacttagagatcactggcatattcaaagggcccctactcggaaaggtgatagccattgatgaggagtctgagacaacactgtccaggcatggtgttgagtttgttaagccctgccaagtgacgggacttgagttcaaagtagtcactattgtgtctgccgcaccaatagaggaaattggccagtccacagctttctacaacgctatcaccaggtcaaagggattgacatatgtccgcgcagggccataggctgaccgctccggtcaattctgaaaaagtgtacatagtattaggtctatcatttgctttagtttcaattacctttctgctttctagaaatagcttaccccacgtcggtgacaacattcacagcttgccacacggaggagcttacagagacggcaccaaagcaatcttgtacaactccccaaatctagggtcacgagtgagtctacacaacggaaagaacgcagcatttgctgccgttttgctactgactttgctgatctatggaagtaaatacatatctcaacgcaatcatacttgtgcttgtggtaacaatcatagcagtcattagcacttccttagtgaggactgaaccttgtgtcatcaagattactggggaatcaatcacagtgttggcttgcaaactagatgcagaaaccataagggccattgccgatctcaagccactctccgttgaacggttaagtttccattgatactcgaaagaggtcagcaccagctagcaacaaacaagaacatggaactgaagaagtccatcagcgattacaccgaggctgagttcaagaagatcatcgaggctatcatcaactgcgagggtgatgagaaaacccaggatgataaccttgagttcttcatcagggtgaccgagtacccttctggtagcgatcttatctactaccctgagggtgataacgatggtagcaccgaggcaattatcaaagaaatcaaggaatggagggctgctaacggtaagcctggttttaagcaagcttaa